European Patent Application EP 4 782 460 A1, published July 29, 2026. Title: peptide fragment and use thereof. Applicant: TOAGOSEI CO., LTD. The sequence listing filed with the application follows.

SEQUENCE LISTING (12 sequences)

SEQ ID NO: 1 - protein, 13 aa, synthetic construct
KKRTLRKSARKKR

SEQ ID NO: 2 - protein, 15 aa, synthetic construct
KKRTLRKSASARKKR

SEQ ID NO: 3 - protein, 15 aa, synthetic construct
KKRTLRKSNSNRKKR

SEQ ID NO: 4 - protein, 15 aa, synthetic construct
KKRTLRKSASNRKKR

SEQ ID NO: 5 - protein, 15 aa, synthetic construct
KKRTLRKSNSARKKR

SEQ ID NO: 6 - protein, 17 aa, synthetic construct
KKRTLRKSNSASARKKR

SEQ ID NO: 7 - protein, 17 aa, synthetic construct
KKRTLRKSASASNRKKR

SEQ ID NO: 8 - protein, 17 aa, synthetic construct
KKRTLRKSNSNSNRKKR

SEQ ID NO: 9 - protein, 19 aa, synthetic construct
KKRTLRKSNSNSNSNRKKR

SEQ ID NO: 10 - protein, 13 aa, synthetic construct
KKRTLRKSNRKKR

SEQ ID NO: 11 - protein, 7 aa, synthetic construct
KKRTLRK

SEQ ID NO: 12 - protein, 4 aa, synthetic construct
RKKR